European Patent Specification EP 3 575 408 B1, published October 1, 2025. Title: 跨膜核酸解旋纳米孔及其构建方法与应用. Applicant: 四川大学. The sequence listing filed with the application follows.

SEQUENCE LISTING (27 sequences)

SEQ ID NO: 1 - protein, 294 aa, Artificial Sequence
  截短体E1-2(306-605)的氨基酸序列
LQTEKFDFGTMVQWAYDHKYAEESKIAYEYALAAGSDSNARAFLATNSQAKHVKDCAMVRHYLRAETQALSMPAYIKARCKLATGEGSWKSILTFFNYQNIELITFINALKLWLKGIPKKNCLAFIGPPNTGKSMLCNSLIHFLGGSVLSFANHKSHFWLASLADTRAALVDDATHACWRYFDTYLRNALDGYPVSIDRKHKAAVQIKAPPLLVTSNIDVQAEDRYLYLHSRVQTFRFEQPCTDESGEQPFNITDADWKSFFVRLWGRLDLIDEEEDSEEDGDSMRTFTCSARN

SEQ ID NO: 2 - DNA, 903 bp, Artificial Sequence
  截短体E1-2(306-605)的编码基因序列
ttgcagaccgagaaattcgacttcggaactatggtgcaatgggcctatgatcacaaatatgctgaagagtctaaaatagcctatgaatatgctttggctgcaggatctgatagcaatgcacgggcttttttagcaactaacagccaagctaagcatgtgaaggactgtgcaactatggtaagacactatctaagagctgaaacacaagcattaagcatgcctgcatatattaaagctaggtgcaagctggcaactggggaaggaagctggaagtctattctaactttttttaattatcagaatattgaattaattacctttattaatgctttaaagctctggctaaaaggaattccaaaaaaaaactgtttagcatttattggccctccaaacacaggcaagtctatgctctgcaactcattaattcattttttgggtggtagtgttttatcttttgccaaccataaaagtcacttttggcttgcttccctagcagatactagagctgctttagtagatgatgctactcatgcttgctggaggtactttgacacatacctcagaaatgcattggatggctaccctgtcagtattgatagaaaacacaaagcagcggttcaaattaaagctccacccctcctggtaaccagtaatattgatgtgcaggcagaggacagatatttgtacttgcatagtcgggtgcaaacctttcgctttgagcagccatgcacagatgaatcgggtgagcaaccttttaatattactgatgcagattggaaatctttttttgtaaggttatgggggcgtttagacctgattgacgaggaggaggatagtgaagaggatggagacagcatgcgaacgtttacatgtagcgcaagaaacacaaatgcagttgattga

SEQ ID NO: 3 - protein, 272 aa, Artificial Sequence
  截短体E1-1(306-577)的氨基酸序列
LQTEKFDFGTMVQWAYDHKYAEESKIAYEYALAAGSDSNARAFLATNSQAKHVKDCATMVRHYLRAETQALSMPAYIKARCKLATGEGSWKSILTFFNYQNIELITFINALKLWLKGIPKKNCLAFIGPPNTGKSMLCNSLIHFLGGSVLSFANHKSHFWLASLADTRAALVDDATHACWRYFDTYLRNALDGYPVSIDRKHKAAVQIKAPPLLVTSNIDVQAEDRYLYLHSRVQTFRFEQPCTDESGEQPFNITDADWKSFFVRLWGRLDL

SEQ ID NO: 4 - DNA, 816 bp, Artificial Sequence
  截短体E1-1(306-577)的编码基因序列
ttgcagaccgagaaattcgacttcggaactatggtgcaatgggcctatgatcacaaatatgctgaggagtctaaaatagcctatgaatatgctttggctgcaggatctgatagcaatgcacgggcttttttagcaactaacagccaagctaagcatgtgaaggactgtgcaactatggtaagacactatctaagagctgaaacacaagcattaagcatgcctgcatatattaaagctaggtgcaagctggcaactggggaaggaagctggaagtctatcctaactttttttaactatcagaatattgaattaattacctttattaatgctttaaagctctggctaaaaggaattccaaaaaaaaactgtttagcatttattggccctccaaacacaggcaagtctatgctctgcaactcattaattcattttttgggtggtagtgttttatcttttgccaaccataaaagtcacttttggcttgcttccctagcagatactagagctgctttagtagatgatgctactcatgcttgctggaggtactttgacacatacctcagaaatgcattggatggctaccctgtcagtattgatagaaaacacaaagcagcggttcaaattaaagctccacccctcctggtaaccagtaatattgatgtgcaggcagaggacagatatttgtacttgcatagtcgggtgcaaacctttcgctttgagcagccatgcacagatgaatcgggtgagcaaccttttaatattactgatgcagattggaaatctttttttgtaaggttatgggggcgtttagacctg

SEQ ID NO: 5 - protein, 605 aa, Artificial Sequence
  野生型牛乳头瘤病毒双链DNA解旋酶E1全长蛋白氨基酸序列
MANDKGSNWDSGLGCSYLLTEAECESDKENEEPGAGVELSVESDRYDSQDEDFVDNASVFQGNHLEVFQALEKKAGEEQILNLKRKVLGSSQNSSGSEASETPVKRRKSGAKRRLFAENEANRVLTPLQVQGEGEGRQELNEEQAISHLHLQLVKSKNATVFKLGLFKSLFLCSFHDITRLFKNDKTTNQQWVLAVFGLAEVFFEASFELLKKQCSFLQMQKRSHEGGTCAVYLICFNTAKSRETVRNLMANMLNVREECLMLQPPKIRGLSAALFWFKSSLSPATLKHGALPEWIRAQTTLNESLQTEKFDFGTMVQWAYDHKYAEESKIAYEYALAAGSDSNARAFLATNSQAKHVKDCATMVRHYLRAETQALSMPAYIKARCKLATGEGSWKSILTFFNYQNIELITFINALKLWLKGIPKKNCLAFIGPPNTGKSMLCNSLIHFLGGSVLSFANHKSHFWLASLADTRAALIDDATHACWRYFDTYLRNALDGYPVSIDRKHKAAVQIKAPPLLVTSNIDVQAEDRYLYLHSRVQTFRFEQPCTDESGEQPFNITDADWKSFFVRLWGRLDLIDEEEDSEEDGDSMRTFTCSARNTNAVD

SEQ ID NO: 6 - protein, 300 aa, Artificial Sequence
  E1-2突变体1（K421L）的氨基酸序列
LQTEKFDFGTMVQWAYDHKYAEESKIAYEYALAAGSDSNARAFLATNSQAKHVKDCATMVRHYLRAETQALSMPAYIKARCKLATGEGSWKSILTFFNYQNIELITFINALKLWLLGIPKKNCLAFIGPPNTGKSMLCNSLIHFLGGSVLSFANHKSHFWLASLADTRAALVDDATHACWRYFDTYLRNALDGYPVSIDRKHKAAVQIKAPPLLVTSNIDVQAEDRYLYLHSRVQTFRFEQPCTDESGEQPFNITDADWKSFFVRLWGRLDLIDEEEDSEEDGDSMRTFTCSARNTNAVD

SEQ ID NO: 7 - protein, 300 aa, Artificial Sequence
  E1-2突变体2（H323W）的氨基酸序列
LQTEKFDFGTMVQWAYDWKYAEESKIAYEYALAAGSDSNARAFLATNSQAKHVKDCATMVRHYLRAETQALSMPAYIKARCKLATGEGSWKSILTFFNYQNIELITFINALKLWLLGIPKKNCLAFIGPPNTGKSMLCNSLIHFLGGSVLSFANHKSHFWLASLADTRAALVDDATHACWRYFDTYLRNALDGYPVSIDRKHKAAVQIKAPPLLVTSNIDVQAEDRYLYLHSRVQTFRFEQPCTDESGEQPFNITDADWKSFFVRLWGRLDLIDEEEDSEEDGDSMRTFTCSARNTNAVD

SEQ ID NO: 8 - DNA, 915 bp, Artificial Sequence
  E1-2突变体1的核苷酸序列
ggatccttgcagaccgagaaattcgacttcggaactatggtgcaatgggcctatgatcacaaatatgctgaggagtctaaaatagcctatgaatatgctttggctgcaggatctgatagcaatgcacgggcttttttagcaactaacagccaagctaagcatgtgaaggactgtgcaactatggtaagacactatctaagagctgaaacacaagcattaagcatgcctgcatatattaaagctaggtgcaagctggcaactggggaaggaagctggaagtctatcctaactttttttaactatcagaatattgaattaattacctttattaatgctttaaagctctggctactgggaattccaaaaaaaaactgtttagcatttattggccctccaaacacaggcaagtctatgctctgcaactcattaattcattttttgggtggtagtgttttatcttttgccaaccataaaagtcacttttggcttgcttccctagcagatactagagctgctttagtagatgatgctactcatgcttgctggaggtactttgacacatacctcagaaatgcattggatggctaccctgtcagtattgatagaaaacacaaagcagcggttcaaattaaagctccacccctcctggtaaccagtaatattgatgtgcaggcagaggacagatatttgtacttgcatagtcgggtgcaaacctttcgctttgagcagccatgcacagatgaatcgggtgagcaaccttttaatattactgatgcagattggaaatctttttttgtaaggttatgggggcgtttagacctgattgacgaggaggaggatagtgaagaggatggagacagcatgcgaacgtttacatgtagcgcaagaaacacaaatgcagttgattaactcgag

SEQ ID NO: 9 - DNA, 912 bp, Artificial Sequence
  E1-2突变体2的核苷酸序列
ggatccttgcagaccgagaaattcgacttcggaactatggtgcaatgggcctatgattggaaatatgctgaggagtctaaaatagcctatgaatatgctttggctgcaggatctgatagcaatgcacgggcttttttagcaactaacagccaagctaagcatgtgaaggactgtgcaactatggtaagacactatctaagagctgaaacacaagcattaagcatgcctgcatatattaaagctaggtgcaagctggcaactggggaaggaagctggaagtctatcctaactttttttaactatcagaatattgaattaattacctttattaatgctttaaagctctggctaggaattccaaaaaaaaactgtttagcatttattggccctccaaacacaggcaagtctatgctctgcaactcattaattcattttttgggtggtagtgttttatcttttgccaaccataaaagtcacttttggcttgcttccctagcagatactagagctgctttagtagatgatgctactcatgcttgctggaggtactttgacacatacctcagaaatgcattggatggctaccctgtcagtattgatagaaaacacaaagcagcggttcaaattaaagctccacccctcctggtaaccagtaatattgatgtgcaggcagaggacagatatttgtacttgcatagtcgggtgcaaacctttcgctttgagcagccatgcacagatgaatcgggtgagcaaccttttaatattactgatgcagattggaaatctttttttgtaaggttatgggggcgtttagacctgattgacgaggaggaggatagtgaagaggatggagacagcatgcgaacgtttacatgtagcgcaagaaacacaaatgcagttgattaactcgag

SEQ ID NO: 10 - DNA, 24 bp, Artificial Sequence
  正向引物
cgggatccttgcagaccgagaaat

SEQ ID NO: 11 - DNA, 46 bp, Artificial Sequence
  反向引物
ccgctcgagttaatgatgatggtgatgatgcaggtctaaacgcccc

SEQ ID NO: 12 - DNA, 53 bp, Artificial Sequence
  正向引物2
agttctgttccaggggcccctgggatccttgcagaccgagaaattcgacttcg

SEQ ID NO: 13 - DNA, 75 bp, Artificial Sequence
  反向引物2
tcagtcagtcacgatgcggccgctcgagttaatcaactgcatttgtgtttcttgcgctacatgtaaacgttcgca

SEQ ID NO: 14 - DNA, 53 bp, Artificial Sequence; identical to SEQ ID NO: 12
  正向引物3

SEQ ID NO: 15 - DNA, 75 bp, Artificial Sequence; identical to SEQ ID NO: 13
  反向引物3

SEQ ID NO: 16 - DNA, 48 bp, Artificial Sequence
  48nt-DNA序列
tttttttttaaaaaattttttggggggttttttccccccttttttttt

SEQ ID NO: 17 - DNA, 44 bp, Artificial Sequence
  44nt-DNA序列
agctccacccctcctggtaaccagtttttttttttttttttttt

SEQ ID NO: 18 - DNA, 44 bp, Artificial Sequence
  44nt-DNA序列1
ttttttttttttttttttttctggttaccaggaggggtggagct

SEQ ID NO: 19 - DNA, 24 bp, Artificial Sequence
  24nt-DNA序列
ctggttaccaggaggggtggagct

SEQ ID NO: 20 - DNA, 22 bp, Artificial Sequence
  带标签的核酸链
cctacgccaccagctccgtagg

SEQ ID NO: 21 - DNA, 42 bp, Artificial Sequence
  带标签的核酸链1
cctacggagctggtggcgtaggtttttttttttttttttttt

SEQ ID NO: 22 - DNA, 22 bp, Artificial Sequence
  带dspacer的双链核酸
tttttttttttttttttttttt

SEQ ID NO: 23 - DNA, 20 bp, Artificial Sequence
  带dspacer的双链核酸1
aaaaaaaaaaaaaaaaaaaa

SEQ ID NO: 24 - DNA, 100 bp, Artificial Sequence
  用于Q-PCR定量转运分析核酸
caggcagaggacagatatttgtacttgcatagtcgggtgcaaacctttcgctttgagcagccatgcacagatgaatcgggtttttttttttttttttttt

SEQ ID NO: 25 - DNA, 80 bp, Artificial Sequence
  用于Q-PCR定量转运分析核酸1
cccgattcatctgtgcatggctgctcaaagcgaaaggtttgcacccgactatgcaagtacaaatatctgtcctctgcctg

SEQ ID NO: 26 - DNA, 20 bp, Artificial Sequence
  用于Q-PCR定量转运引物1
caggcagaggacagatattt

SEQ ID NO: 27 - DNA, 20 bp, Artificial Sequence
  用于Q-PCR定量转运引物2
cccgattcatctgtgcatgg